European Patent Application EP 4 261 280 A1, published October 18, 2023. Title: 氨基酸脱氢酶突变体及其应用. Applicant: 凯莱英生命科学技术（天津）有限公司. The sequence listing filed with the application follows.

SEQUENCE LISTING (2 sequences)

SEQ ID NO: 1 - protein, 368 aa, Thermoactinomyces intermedius ATCC33205
MRDVFEMMDRYGHEQVIFCRHPQTGLKAIIALHNTTAGPALGGCRMIPYASTDEALEDVLRLSKGMTYKCSLADVDFGGGKMVIIGDPKKDKSPELFRVIGRFVGGLNGRFYTGTDMGTNPEDFVHAARESKSFLGLPKSYGGKGDTSIPTALGVFHGMRATARFLWGTDQLKGRVVAIQGVGKVGERLLQLLVEVGAYCKIADIDSVRCEQLKEKYGDKVQLVDVNRIHKESCDIFSPCAKGGVVNDDTIDEFRCLAIVGSANNQLVEDRHGALLQKRSICYAPDYLVNAGGLIQVADELEGFHEERVLAKTEAIYDMVLDIFHRAKNENITTCEAADRIVMERLKKLTDIRRILLEDPRNSARRLE

SEQ ID NO: 2 - DNA, 1107 bp, Thermoactinomyces intermedius ATCC33205
atgcgtgacgtattcgaaatgatggatcgctacggccacgagcaggtgattttctgtcgtcatccgcagactggcctgaaagcgatcatcgctctgcataacaccactgccggtccggcactgggcggttgtcgcatgattccatacgcaagcaccgatgaagctctggaagacgttctgcgtctgagcaaaggtatgacctataaatgctctctggcggatgttgatttcggtggcggtaaaatggtgattatcggcgatccgaaaaaggataaaagcccagaactgttccgtgttatcggtcgcttcgttggcggcctgaacggtcgtttctataccggtactgatatgggcaccaatccggaagatttcgtgcacgccgctcgcgaaagcaaatcttttctaggtctgcctaaatcttacggtggtaaaggtgacacttctatcccgaccgcactgggtgtatttcacggcatgcgcgcgaccgcccgctttctgtggggcaccgatcaactgaaaggtcgtgttgttgctatccagggtgttggcaaagtgggtgaacgtctgctgcagctgctggtggaagtgggtgcatactgcaaaattgctgatattgactctgtacgttgtgagcagctgaaagaaaagtacggcgacaaagtccagctggtagacgtgaaccgtatccacaaagagtcttgtgacatcttctccccgtgcgcaaaaggcggcgtagtcaacgacgacactattgacgaattccgctgcctggcgattgttggttccgcgaacaatcagctggttgaagatcgtcatggcgcgctgctgcaaaaacgctccatttgctatgccccggattatctggttaacgctggcggtctgatccaggtcgcagacgaactggagggttttcacgaggagcgtgtgctggcgaaaacggaagccatctacgacatggttctggacatcttccaccgcgctaagaacgaaaacatcactacctgcgaagcagcggaccgtatcgtaatggaacgtctgaagaagctgacggacatccgtcgtatcctgctggaagatccgcgtaactccgcgcgtcgtctcgagtga